European Patent Application EP 4 458 852 A1, published November 6, 2024. Title: ANTI-βKLOTHO ANTIBODY AND USE THEREOF. Applicant: SHANGHAI JMT-BIO TECHNOLOGY CO., LTD. Application EP 22914995.0, filed December 29, 2022. The sequence listing filed with the application follows.

SEQUENCE LISTING (52 sequences)

SEQ ID NO: 1 - protein, 5 aa, synthetic construct
SYGIS

SEQ ID NO: 2 - protein, 17 aa, synthetic construct
WISAYNGNTNYAQKLQG

SEQ ID NO: 3 - protein, 9 aa, synthetic construct
LYGSGSLYY

SEQ ID NO: 4 - protein, 11 aa, synthetic construct
QASQDIRNYIN

SEQ ID NO: 5 - protein, 7 aa, synthetic construct
AASSLQS

SEQ ID NO: 6 - protein, 10 aa, synthetic construct
QQSYSTPQWT

SEQ ID NO: 7 - protein, 8 aa, synthetic construct
GYTFTSYG

SEQ ID NO: 8 - protein, 8 aa, synthetic construct
ISAYNGNT

SEQ ID NO: 9 - protein, 11 aa, synthetic construct
ATLYGSGSLYY

SEQ ID NO: 10 - protein, 6 aa, synthetic construct
QDIRNY

SEQ ID NO: 11 - protein, 11 aa, synthetic construct
QASQDIRNYIN

SEQ ID NO: 12 - protein, 118 aa, synthetic construct
EVQLVQSGAEVKKPGASVKVSCKASGYTFTSYGISWVRQAPGQGLEWMGWISAYNGNTNYAQKLQGRVTMTTDTSTSTAYMELRSLRSDDTAVYYCATLYGSGSLYYWGQGTLVTVSS

SEQ ID NO: 13 - protein, 108 aa, synthetic construct
DIVMTQSPSSLSAPVGDRVTITCQASQDIRNYINWFQQKPGKAPKLLIYAASSLQSGVPSRFSGSGSGTDFTLTISSLQPEDFATYYCQQSYSTPQWTFGQGTKVEIK

SEQ ID NO: 14 - protein, 17 aa, synthetic construct
WISAYNGRTNYAQKLQG

SEQ ID NO: 15 - protein, 7 aa, synthetic construct
AASRLQS

SEQ ID NO: 16 - protein, 8 aa, synthetic construct
GYRFTSYG

SEQ ID NO: 17 - protein, 8 aa, synthetic construct
ISAYNGRT

SEQ ID NO: 18 - protein, 118 aa, synthetic construct
EVQLVQSGAEVKKPGASVKVSCKASGYRFTSYGISWVRQAPGQGLEWMGWISAYNGRTNYAQKLQGRVTMTTDTSTSTAYMELRSLRSDDTAVYYCATLYGSGSLYYWGQGTLVTVSS

SEQ ID NO: 19 - protein, 108 aa, synthetic construct
DIVMTQSPSSLSAPVGDRVTITCQASQDIRNYINWFQQKPGKAPKLLIYAASRLQSGVPSRFSGSGSGTDFTLTISSLQPEDFATYYCQQSYSTPQWTFGQGTKVEIK

SEQ ID NO: 20 - protein, 17 aa, synthetic construct
WISAYTGNTNYAQKLQG

SEQ ID NO: 21 - protein, 7 aa, synthetic construct
AASSRQS

SEQ ID NO: 22 - protein, 8 aa, synthetic construct
GYTFRSYG

SEQ ID NO: 23 - protein, 8 aa, synthetic construct
ISAYTGNT

SEQ ID NO: 24 - protein, 118 aa, synthetic construct
EVQLVQSGAEVKKPGASVKVSCKASGYTFRSYGISWVRQAPGQGLEWMGWISAYTGNTNYAQKLQGRVTMTTDTSTSTAYMELRSLRSDDTAVYYCATLYGSGSLYYWGQGTLVTVSS

SEQ ID NO: 25 - protein, 108 aa, synthetic construct
DIVMTQSPSSLSAPVGDRVTITCQASQDIRNYINWFQQKPGKAPKLLIYAASSRQSGVPSRFSGSGSGTDFTLTISSLQPEDFATYYCQQSYSTPQWTFGQGTKVEIK

SEQ ID NO: 26 - protein, 5 aa, synthetic construct
SGGIS

SEQ ID NO: 27 - protein, 7 aa, synthetic construct
AASFLQS

SEQ ID NO: 28 - protein, 8 aa, synthetic construct
GYTFTSGG

SEQ ID NO: 29 - protein, 118 aa, synthetic construct
EVQLVQSGAEVKKPGASVKVSCKASGYTFTSGGISWVRQAPGQGLEWMGWISAYNGRTNYAQKLQGRVTMTTDTSTSTAYMELRSLRSDDTAVYYCATLYGSGSLYYWGQGTLVTVSS

SEQ ID NO: 30 - protein, 108 aa, synthetic construct
DIVMTQSPSSLSAPVGDRVTITCQASQDIRNYINWFQQKPGKAPKLLIYAASFLQSGVPSRFSGSGSGTDFTLTISSLQPEDFATYYCQQSYSTPQWTFGQGTKVEIK

SEQ ID NO: 31 - protein, 9 aa, synthetic construct
LLPSGSLYY

SEQ ID NO: 32 - protein, 11 aa, synthetic construct
ATLLPSGSLYY

SEQ ID NO: 33 - protein, 118 aa, synthetic construct
EVQLVQSGAEVKKPGASVKVSCKASGYTFTSYGISWVRQAPGQGLEWMGWISAYNGNTNYAQKLQGRVTMTTDTSTSTAYMELRSLRSDDTAVYYCATLLPSGSLYYWGQGTLVTVSS

SEQ ID NO: 34 - protein, 7 aa, synthetic construct
AASGLQS

SEQ ID NO: 35 - protein, 8 aa, synthetic construct
GYTFKSYG

SEQ ID NO: 36 - protein, 118 aa, synthetic construct
EVQLVQSGAEVKKPGASVKVSCKASGYTFKSYGISWVRQAPGQGLEWMGWISAYNGRTNYAQKLQGRVTMTTDTSTSTAYMELRSLRSDDTAVYYCATLYGSGSLYYWGQGTLVTVSS

SEQ ID NO: 37 - protein, 108 aa, synthetic construct
DIVMTQSPSSLSAPVGDRVTITCQASQDIRNYINWFQQKPGKAPKLLIYAASGLQSGVPSRFSGSGSGTDFTLTISSLQPEDFATYYCQQSYSTPQWTFGQGTKVEIK

SEQ ID NO: 38 - protein, 17 aa, synthetic construct
WISAYSGNTNYAQKLQG

SEQ ID NO: 39 - protein, 8 aa, synthetic construct
GYAFTSYG

SEQ ID NO: 40 - protein, 8 aa, synthetic construct
ISAYSGNT

SEQ ID NO: 41 - protein, 118 aa, synthetic construct
EVQLVQSGAEVKKPGASVKVSCKASGYAFTSYGISWVRQAPGQGLEWMGWISAYSGNTNYAQKLQGRVTMTTDTSTSTAYMELRSLRSDDTAVYYCATLYGSGSLYYWGQGTLVTVSS

SEQ ID NO: 42 - protein, 7 aa, synthetic construct
AASYLQS

SEQ ID NO: 43 - protein, 118 aa, synthetic construct
EVQLVQSGAEVKKPGASVKVSCKASGYTFTSYGISWVRQAPGQGLEWMGWISAYSGNTNYAQKLQGRVTMTTDTSTSTAYMELRSLRSDDTAVYYCATLYGSGSLYYWGQGTLVTVSS

SEQ ID NO: 44 - protein, 108 aa, synthetic construct
DIVMTQSPSSLSAPVGDRVTITCQASQDIRNYINWFQQKPGKAPKLLIYAASYLQSGVPSRFSGSGSGTDFTLTISSLQPEDFATYYCQQSYSTPQWTFGQGTKVEIK

SEQ ID NO: 45 - protein, 7 aa, synthetic construct
AASHLQS

SEQ ID NO: 46 - protein, 8 aa, synthetic construct
GYLFTSYG

SEQ ID NO: 47 - protein, 118 aa, synthetic construct
EVQLVQSGAEVKKPGASVKVSCKASGYLFTSYGISWVRQAPGQGLEWMGWISAYTGNTNYAQKLQGRVTMTTDTSTSTAYMELRSLRSDDTAVYYCATLYGSGSLYYWGQGTLVTVSS

SEQ ID NO: 48 - protein, 108 aa, synthetic construct
DIVMTQSPSSLSAPVGDRVTITCQASQDIRNYINWFQQKPGKAPKLLIYAASHLQSGVPSRFSGSGSGTDFTLTISSLQPEDFATYYCQQSYSTPQWTFGQGTKVEIK

SEQ ID NO: 49 - protein, 118 aa, synthetic construct
EVQLVQSGAEVKKPGASVKVSCKASGYTFTSYGISWVRQAPGQGLEWMGWISAYSGNTNYAQKLQGRVTMTTDTSTSTAYMELRSLRSDDTAVYYCATLLPSGSLYYWGQGTLVTVSS

SEQ ID NO: 50 - protein, 330 aa, synthetic construct
ASTKGPSVFPLAPSSKSTSGGTAALGCLVKDYFPEPVTVSWNSGALTSGVHTFPAVLQSSGLYSLSSVVTVPSSSLGTQTYICNVNHKPSNTKVDKKVEPKSCDKTHTCPPCPAPALAGGPSVFLFPPKPKDTLMISRTPEVTCVVVDVSHEDPEVKFNWYVDGVEVHNAKTKPREEQYNSTYRVVSVLTVLHQDWLNGKEYKCKVSNKALPAPIEKTISKAKGQPREPQVYTLPPSREEMTKNQVSLTCLVKGFYPSDIAVEWESNGQPENNYKTTPPVLDSDGSFFLYSKLTVDKSRWQQGNVFSCSVMHEALHNHYTQKSLSLSPGK

SEQ ID NO: 51 - protein, 107 aa, synthetic construct [sequence omitted]

SEQ ID NO: 52 - protein, 1044 aa, Homo sapiens
MKPGCAAGSPGNEWIFFSTDEITTRYRNTMSNGGLQRSVILSALILLRAVTGFSGDGRAIWSKNPNFTPVNESQLFLYDTFPKNFFWGIGTGALQVEGSWKKDGKGPSIWDHFIHTHLKNVSSTNGSSDSYIFLEKDLSALDFIGVSFYQFSISWPRLFPDGIVTVANAKGLQYYSTLLDALVLRNIEPIVTLYHWDLPLALQEKYGGWKNDTIIDIFNDYATYCFQMFGDRVKYWITIHNPYLVAWHGYGTGMHAPGEKGNLAAVYTVGHNLIKAHSKVWHNYNTHFRPHQKGWLSITLGSHWIEPNRSENTMDIFKCQQSMVSVLGWFANPIHGDGDYPEGMRKKLFSVLPIFSEAEKHEMRGTADFFAFSFGPNNFKPLNTMAKMGQNVSLNLREALNWIKLEYNNPRILIAENGWFTDSRVKTEDTTAIYMMKNFLSQVLQAIRLDEIRVFGYTAWSLLDGFEWQDAYTIRRGLFYVDFNSKQKERKPKSSAHYYKQIIRENGFSLKESTPDVQGQFPCDFSWGVTESVLKPESVASSPQFSDPHLYVWNATGNRLLHRVEGVRLKTRPAQCTDFVNIKKQLEMLARMKVTHYRFALDWASVLPTGNLSAVNRQALRYYRCVVSEGLKLGISAMVTLYYPTHAHLGLPEPLLHADGWLNPSTAEAFQAYAGLCFQELGDLVKLWITINEPNRLSDIYNRSGNDTYGAAHNLLVAHALAWRLYDRQFRPSQRGAVSLSLHADWAEPANPYADSHWRAAERFLQFEIAWFAEPLFKTGDYPAAMREYIASKHRRGLSSSALPRLTEAERRLLKGTVDFCALNHFTTRFVMHEQLAGSRYDSDRDIQFLQDITRLSSPTRLAVIPWGVRKLLRWVRRNYGDMDIYITASGIDDQALEDDRLRKYYLGKYLQEVLKAYLIDKVRIKGYYAFKLAEEKSKPRFGFFTSDFKAKSSIQFYNKVISSRGFPFENSSSRCSQTQENTECTVCLFLVQKKPLIFLGCCFFSTLVLLLSIAIFQRQKRRKFWKAKNLQHIPLKKGKRVVS